European Patent Specification EP 3 448 426 B1, published May 28, 2025. Title: Methods for Treating Patients with Familial Hypercholesterolemia. Applicant: Regeneron Pharmaceuticals, Inc. The sequence listing filed with the application follows.

SEQUENCE LISTING (9 sequences)

SEQ ID NO: 1 - protein, 126 aa, Artificial Sequence
  HCVR
EVQLVESGGGVIQPGGSLRLSCAASGFTFDDYAMNWVRQGPGKGLEWVSAISGDGGSTYYADSVKGRFTISRDNSKNSLYLQMNSLRAEDTAFFYCAKDLRNTIFGVVIPDAFDIWGQGTMVTVSS

SEQ ID NO: 2 - protein, 8 aa, Artificial Sequence
  HCDR1
GFTFDDYA

SEQ ID NO: 3 - protein, 8 aa, Artificial Sequence
  HCDR2
ISGDGGST

SEQ ID NO: 4 - protein, 19 aa, Artificial Sequence
  HCDR3
AKDLRNTIFGVVIPDAFDI

SEQ ID NO: 5 - protein, 108 aa, Artificial Sequence
  LCVR
DIQMTQSPSTLSASVGDRVTITCRASQSIRSWLAWYQQKPGKAPKLLIYKASSLESGVPSRFSGSGSGTEFTLTISSLQPDDFATYYCQQYNSYSYTFGQGTKLEIKR

SEQ ID NO: 6 - protein, 6 aa, Artificial Sequence
  LCDR1
QSIRSW

SEQ ID NO: 7 - protein, 3 aa, Artificial Sequence
  LCDR2
KAS

SEQ ID NO: 8 - protein, 9 aa, Artificial Sequence
  LCDR3
QQYNSYSYT

SEQ ID NO: 9 - protein, 432 aa, Artificial Sequence
  hANGPTL3
MFTIKLLLFIVPLVISSRIDQDNSSFDSLSPEPKSRFAMLDDVKILANGLLQLGHGLKDFVHKTKGQINDIFQKLNIFDQSFYDLSLQTSEIKEEEKELRRTTYKLQVKNEEVKNMSLELNSKLESLLEEKILLQQKVKYLEEQLTNLIQNQPETPEHPEVTSLKTFVEKQDNSIKDLLQTVEDQYKQLNQQHSQIKEIENQLRRTSIQEPTEISLSSKPRAPRTTPFLQLNEIRNVKHDGIPAECTTIYNRGEHTSGMYAIRPSNSQVFHVYCDVISGSPWTLIQHRIDGSQNFNETWENYKYGFGRLDGEFWLGLEKIYSIVKQSNYVLRIELEDWKDNKHYIEYSFYLGNHETNYTLHLVAITGNVPNAIPENKDLVFSTWDHKAKGHFNCPEGYSGGWWWHDECGENNLNGKYNKPRAKSKPERRRGL